European Patent Specification EP 3 720 274 B1, published February 19, 2025. Title: bZIP TRANSCRIPTION FACTORS REGULATE CONVERSION OF NICOTINE TO NORNICOTINE. Applicant: University of Kentucky Research Foundation. The sequence listing filed with the application follows.

SEQUENCE LISTING (6 sequences)

SEQ ID NO: 1 - DNA, 435 bp, Nicotiana tabacum
atggctttgacacagcaaccggctagttcaggttctgatggccaacgttatgccacaaatgacgatagaaaacgaaagagaatggagtccaaccgtgaatctgcaaggcggtcacggatgagaaagcagcagcatttggaggagttgatgagccaaatgacacagctacagaatcagaacgttctgtggcgcgagaagattgatgctgtgggaagaaactacctcaccctcgatgcggagaacaatgtcttgagggctcaaatggcagaactgactgaacgcttggattctctcaattcgctcactcgtttctgggctgatgctaatggactagctgtggatatccctgaaattcctgacactttgcttgagccctggcagcttccttgcccaattcaacccatcactgcttctgctgatatgtttcagttttga

SEQ ID NO: 2 - protein, 144 aa, Nicotiana tabacum
NALTQQPASSGSDGQRYATNDDRKRKRMESNRESARRSRMRKQQHLEELMSQMTQLQNQNVLWREKIDAVGRNYLTLDAENNVLRAQMAELTERLDSLNSLTRFWADANGLAVDIPEIPDTLLEPWQLPCPIQPITASADMFQF

SEQ ID NO: 3 - DNA, 435 bp, Nicotiana tabacum
atggcttcgatacagcaaccagctagttcaggttctgatggccaacgatatgctatgaacgacgatagaaaacgaaagagaatggagtccaaccgtgaatctgcaaggcggtcacggatgaggaagcagcagcatttggaagagttgatgagccaaatgacacagctacagaatcagaacgttctgtggcgtgagaagattgatgctgtgggaagaaactacctgacccttgatgcggagaacaatgtcctgagggctcaaatggcagaactgactgaacgcttggattcgctcaattcgctcgctcgtttctgggctgatgctaatggactagctgtggatatccctgaaattccagacactttgcttgagccgtggcagcttccttgcccaattcaacccatcactgcttctgctaatatgtttcagttttga

SEQ ID NO: 4 - protein, 144 aa, Nicotiana tabacum
NASIQQPASSGSDGQRYAMNDDRKRKRMESNRESARRSRMRKQQHLEELMSQMTQLQNQNVLWREKIDAVGRNYLTLDAENNVLRAQMAELTERLDSLNSLARFWADANGLAVDIPEIPDTLLEPWQLPCPIQPITASANMFQF

SEQ ID NO: 5 - protein, 455 aa, Nicotiana tabacum
MDRVFSVDDDIGDHFWSTPPTADLGVDSPTAAAAVSYSKMMNRSSSEWAFQRFLQEATAAGTSTSSPPQPPTMTASSSSSSHQNDVVEIKDENLSIPNLNPSTALNSKPASSFGLAPPPNIAVDSEEYQAFLKSQLHLACAAVALTRGKSLNPQDSGSTAHDKGSETASAAQSGSHVSTLGKCYLRSGQEVAKIQDKDAGGPVGIPSLPPVQKKPVVQVRSTTSGSSREQSDDDEAEGEAETTQGMDPADAKRVRRMLSNRESARRSRRRKQAHLTELETQVSQLRVENSSLLKRLTDISQKYNEAAVDNRVLKADVETLRAKVKMAEETVKRVTGLNPLFQAMSEISSMVMPSYSGSPSDTSADAAVPVQDDPKHHYYQQPPNNLMPTHDPRIQNGMVDVPPIENVEQNPATAAVGGNKMGRTTSMQRVASLEHLQKRIRGEVSSCGTQGRGEQ

SEQ ID NO: 6 - protein, 442 aa, Nicotiana tabacum
MDRVFSVDDDIGDHFWSTPPTADLGVDSPTTATAASYSKMMNRSSSEWAFQRFLQEATAAGTSTSSHPQPPTMTASSSSSSHQNDVVEIKDENLSTPNLNPSTALNSKPASSFGLTPPPNIAVDSEEYQAFLKSQLHLACAAVALTRGKSLNPQDSGSTAHDKGSETASAAQSGSHEMAKIQDKDAGGPVGIPSLPPVQKKPVVQVRSTTSGSSREQSDDDEAEGEAETTQGMDPADAKRVRRMLSNRESARRSRRRKQAHLTELETQVSQLRVENSSLLKRLTDISQKYNEAAVDNRVLKADVETLRAKVKMAEETVKRVTGLNPLFQAMSEISSMVMPSYSGSPSDTSADAAVPVQDDPKHHYYQQPPNNHMPTNDPRIQNGMVDVPPIENVQQNPATAAVGGNKMGRTASMQRVASLEHLQKRIRGEISSCGTQGRGEQ